European Patent Specification EP 3 836 887 B1, published July 17, 2024. Title: PARTICLE-CONTAINING DROPLET SYSTEMS WITH MONODISPERSE FLUID VOLUMES. Applicant: The Regents of the University of California. Application PCT/US19/46835. The sequence listing filed with the application follows.

SEQUENCE LISTING (2 sequences)

SEQ ID NO: 1 - protein, 10 aa, Artificial Sequence
  cell adhesion peptide
RGDSPGERCG

SEQ ID NO: 2 - protein, 16 aa, Artificial Sequence
  crosslinker peptide
GCRDGPQGIWGQDRCG